European Patent Specification EP 4 139 485 B1, published September 6, 2023. Title: METHODS FOR SPATIAL ANALYSIS USING TARGETED RNA DEPLETION. Applicant: 10x Genomics, Inc. and Spatial Transcriptomics AB. The sequence listing filed with the application follows.

SEQUENCE LISTING (195 sequences)

SEQ ID NO: 1 - DNA, 50 bp, Artificial
  Synthetic probe AG9327_18_1
taatgatccttccgcaggttcacctacggaaaccttgttacgacttttac

SEQ ID NO: 2 - DNA, 50 bp, Artificial
  Synthetic probe AG9328_18_2
ttcctctagatagtcaagttcgaccgtcttctcagcgctccgccagggcc

SEQ ID NO: 3 - DNA, 50 bp, Artificial
  Synthetic probe AG9329_18_3
gtgggccgaccccggcggggccgatccgagggcctcactaaaccatccaa

SEQ ID NO: 4 - DNA, 50 bp, Artificial
  Synthetic probe AG9330_18_4
tcggtagtagcgacgggcggtgtgtacaaagggcagggacttaatcaacg

SEQ ID NO: 5 - DNA, 50 bp, Artificial
  Synthetic probe AG9331_18_5
caagcttatgacccgcacttactcgggaattccctcgttcatggggaata

SEQ ID NO: 6 - DNA, 50 bp, Artificial
  Synthetic probe AG9332_18_6
attgcaatccccgatccccatcacgaatggggttcaacgggttacccgcg

SEQ ID NO: 7 - DNA, 50 bp, Artificial
  Synthetic probe AG9333_18_7
cctgccggcgtagggtaggcacacgctgagccagtcagtgtagcgcgcgt

SEQ ID NO: 8 - DNA, 50 bp, Artificial
  Synthetic probe AG9334_18_8
gcagccccggacatctaagggcatcacagacctgttattgctcaatctcg

SEQ ID NO: 9 - DNA, 50 bp, Artificial
  Synthetic probe AG9335_18_9
ggtggctgaacgccacttgtccctctaagaagttgggggacgccgaccgc

SEQ ID NO: 10 - DNA, 50 bp, Artificial
  Synthetic probe AG9336_18_10
tcgggggtcgcgtaactagttagcatgccagagtctcgttcgttatcgga

SEQ ID NO: 11 - DNA, 50 bp, Artificial
  Synthetic probe AG9337_18_11
attaaccagacaaatcgctccaccaactaagaacggccatgcaccaccac

SEQ ID NO: 12 - DNA, 50 bp, Artificial
  Synthetic probe AG9338_18_12
ccacggaatcgagaaagagctatcaatctgtcaatcctgtccgtgtccgg

SEQ ID NO: 13 - DNA, 50 bp, Artificial
  Synthetic probe AG9339_18_13
gccgggtgaggtttcccgtgttgagtcaaattaagccgcaggctccactc

SEQ ID NO: 14 - DNA, 50 bp, Artificial
  Synthetic probe AG9340_18_14
ctggtggtgcccttccgtcaattcctttaagtttcagctttgcaaccata

SEQ ID NO: 15 - DNA, 50 bp, Artificial
  Synthetic probe AG9341_18_15
ctccccccggaacccaaagactttggtttcccggaagctgcccggcgggt

SEQ ID NO: 16 - DNA, 50 bp, Artificial
  Synthetic probe AG9342_18_16
catgggaataacgccgccgcatcgccggtcggcatcgtttatggtcggaa

SEQ ID NO: 17 - DNA, 50 bp, Artificial
  Synthetic probe AG9343_18_17
ctacgacggtatctgatcgtcttcgaacctccgactttcgttcttgatta

SEQ ID NO: 18 - DNA, 50 bp, Artificial
  Synthetic probe AG9344_18_18
atgaaaacattcttggcaaatgctttcgctctggtccgtcttgcgccggt

SEQ ID NO: 19 - DNA, 50 bp, Artificial
  Synthetic probe AG9345_18_19
ccaagaatttcacctctagcggcgcaatacgaatgcccccggccgtccct

SEQ ID NO: 20 - DNA, 50 bp, Artificial
  Synthetic probe AG9346_18_20
cttaatcatggcctcagttccgaaaaccaacaaaatagaaccgcggtcct

SEQ ID NO: 21 - DNA, 50 bp, Artificial
  Synthetic probe AG9347_18_21
attccattattcctagctgcggtatccaggcggctcgggcctgctttgaa

SEQ ID NO: 22 - DNA, 50 bp, Artificial
  Synthetic probe AG9348_18_22
cactctaattttttcaaagtaaacgcttcgggccccgcgggacactcagc

SEQ ID NO: 23 - DNA, 50 bp, Artificial
  Synthetic probe AG9349_18_23
taagagcatcgagggggcgccgagaggcaaggggcggggacgggcggtgg

SEQ ID NO: 24 - DNA, 50 bp, Artificial
  Synthetic probe AG9350_18_24
ctcgcctcgcggcggaccgcccgcccgctcccaagatccaactacgagct

SEQ ID NO: 25 - DNA, 50 bp, Artificial
  Synthetic probe AG9351_18_25
ttttaactgcagcaactttaatatacgctattggagctggaattaccgcg

SEQ ID NO: 26 - DNA, 50 bp, Artificial
  Synthetic probe AG9352_18_26
gctgctggcaccagacttgccctccaatggatcctcgttaaaggatttaa

SEQ ID NO: 27 - DNA, 50 bp, Artificial
  Synthetic probe AG9353_18_27
agtggactcattccaattacagggcctcgaaagagtcctgtattgttatt

SEQ ID NO: 28 - DNA, 50 bp, Artificial
  Synthetic probe AG9354_18_28
tttcgtcactacctccccgggtcgggagtgggtaatttgcgcgcctgctg

SEQ ID NO: 29 - DNA, 50 bp, Artificial
  Synthetic probe AG9355_18_29
ccttccttggatgtggtagccgtttctcaggctccctctccggaatcgaa

SEQ ID NO: 30 - DNA, 50 bp, Artificial
  Synthetic probe AG9356_18_30
ccctgattccccgtcacccgtggtcaccatggtaggcacggcgactacca

SEQ ID NO: 31 - DNA, 48 bp, Artificial
  Synthetic probe AG9357_18_31
tcgaaagttgatagggcagacgttcgaatgggtcgtcgccgccacggg

SEQ ID NO: 32 - DNA, 50 bp, Artificial
  Synthetic probe AG9358_18_32
gcgtgcgatcggcccgaggttatctagagtcaccaaagccgccggcgccc

SEQ ID NO: 33 - DNA, 50 bp, Artificial
  Synthetic probe AG9359_18_33
gccccccggccggggccggagaggggctgaccgggttggttttgatctga

SEQ ID NO: 34 - DNA, 50 bp, Artificial
  Synthetic probe AG9360_18_34
taaatgcacgcatcccccccgcgaagggggtcagcgcccgtcggcatgta

SEQ ID NO: 35 - DNA, 50 bp, Artificial
  Synthetic probe AG9361_18_35
ttagctctagaattaccacagttatccaagtaggagaggagcgagcgacc

SEQ ID NO: 36 - DNA, 50 bp, Artificial
  Synthetic probe AG9362_18_36
aaaggaaccataactgatttaatgagccattcgcagtttcactgtaccgg

SEQ ID NO: 37 - DNA, 50 bp, Artificial
  Synthetic probe AG9363_18_37
ccgtgcgtacttagacatgcatggcttaatctttgagacaagcatatgct

SEQ ID NO: 38 - DNA, 50 bp, Artificial
  Synthetic probe AG9364_18_38
tggcttaatctttgagacaagcatatgctactggcaggatcaaccaggta

SEQ ID NO: 39 - DNA, 50 bp, Artificial
  Synthetic probe AG9365_28_1
gacaaacccttgtgtcgagggctgactttcaatagatcgcagcgagggag

SEQ ID NO: 40 - DNA, 50 bp, Artificial
  Synthetic probe AG9366_28_2
ctgctctgctacgtacgaaaccccgacccagaagcaggtcgtctacgaat

SEQ ID NO: 41 - DNA, 49 bp, Artificial
  Synthetic probe AG9367_28_3
ggtttagcgccaggttccccacgaacgtgcggtgcgtgacgggcgaggg

SEQ ID NO: 42 - DNA, 50 bp, Artificial
  Synthetic probe AG9368_28_4
gcggccgcctttccggccgcgccccgtttcccaggacgaagggcactccg

SEQ ID NO: 43 - DNA, 50 bp, Artificial
  Synthetic probe AG9369_28_5
caccggaccccggtcccggcgcgcggcggggcacgcgccctcccgcggcg

SEQ ID NO: 44 - DNA, 49 bp, Artificial
  Synthetic probe AG9370_28_6
gggcgcgtggagggggggcggcccgccggcggggacaggcgggggaccg

SEQ ID NO: 45 - DNA, 50 bp, Artificial
  Synthetic probe AG9371_28_7
gctatccgaggccaaccgaggctccgcggcgctgccgtatcgttcgcctg

SEQ ID NO: 46 - DNA, 50 bp, Artificial
  Synthetic probe AG9372_28_8
ggcgggattctgacttagaggcgttcagtcataatcccacagatggtagc

SEQ ID NO: 47 - DNA, 50 bp, Artificial
  Synthetic probe AG9373_28_9
ttcgccccattggctcctcagccaagcacatacaccaaatgtctgaacct

SEQ ID NO: 48 - DNA, 50 bp, Artificial
  Synthetic probe AG9374_28_10
gcggttcctctcgtactgagcaggattaccatggcaacaacacatcatca

SEQ ID NO: 49 - DNA, 50 bp, Artificial
  Synthetic probe AG9375_28_11
gtagggtaaaactaacctgtctcacgacggtctaaacccagctcacgttc

SEQ ID NO: 50 - DNA, 50 bp, Artificial
  Synthetic probe AG9376_28_12
cctattagtgggtgaacaatccaacgcttggcgaattctgcttcacaatg

SEQ ID NO: 51 - DNA, 50 bp, Artificial
  Synthetic probe AG9377_28_13
ataggaagagccgacatcgaaggatcaaaaagcgacgtcgctatgaacgc

SEQ ID NO: 52 - DNA, 50 bp, Artificial
  Synthetic probe AG9378_28_14
ttggccgccacaagccagttatccctgtggtaacttttctgacacctcct

SEQ ID NO: 53 - DNA, 50 bp, Artificial
  Synthetic probe AG9379_28_15
gcttaaaacccaaaaggtcagaaggatcgtgaggccccgctttcacggtc

SEQ ID NO: 54 - DNA, 50 bp, Artificial
  Synthetic probe AG9380_28_16
tgtattcgtactgaaaatcaagatcaagcgagcttttgcccttctgctcc

SEQ ID NO: 55 - DNA, 50 bp, Artificial
  Synthetic probe AG9381_28_17
acgggaggtttctgtcctccctgagctcgccttaggacacctgcgttacc

SEQ ID NO: 56 - DNA, 50 bp, Artificial
  Synthetic probe AG9382_28_18
gtttgacaggtgtaccgccccagtcaaactccccacctggcactgtcccc

SEQ ID NO: 57 - DNA, 50 bp, Artificial
  Synthetic probe AG9383_28_19
ggagcgggtcgcgcccggccgggcgggcgcttggcgccagaagcgagagc

SEQ ID NO: 58 - DNA, 50 bp, Artificial
  Synthetic probe AG9384_28_20
ccctcgggctcgcccccccgcctcaccgggtcagtgaaaaaacgatcaga

SEQ ID NO: 59 - DNA, 50 bp, Artificial
  Synthetic probe AG9385_28_21
gtagtggtatttcaccggcggcccgcagggccgcggaccccgccccgggc

SEQ ID NO: 60 - DNA, 49 bp, Artificial
  Synthetic probe AG9386_28_22
ccctcgcggggacaccggggggcgccgggggcctcccacttattctaca

SEQ ID NO: 61 - DNA, 50 bp, Artificial
  Synthetic probe AG9387_28_23
cctctcatgtctcttcaccgtgccagactagagtcaagctcaacagggtc

SEQ ID NO: 62 - DNA, 50 bp, Artificial
  Synthetic probe AG9388_28_24
ttctttccccgctgattccgccaagcccgttcccttggctgtggtttcgc

SEQ ID NO: 63 - DNA, 50 bp, Artificial
  Synthetic probe AG9389_28_25
tggatagtaggtagggacagtgggaatctcgttcatccattcatgcgcgt

SEQ ID NO: 64 - DNA, 50 bp, Artificial
  Synthetic probe AG9390_28_26
cactaattagatgacgaggcatttggctaccttaagagagtcatagttac

SEQ ID NO: 65 - DNA, 50 bp, Artificial
  Synthetic probe AG9391_28_27
tcccgccgtttacccgcgcttcattgaatttcttcactttgacattcaga

SEQ ID NO: 66 - DNA, 50 bp, Artificial
  Synthetic probe AG9392_28_28
gcactgggcagaaatcacatcgcgtcaacacccgccgcgggccttcgcga

SEQ ID NO: 67 - DNA, 50 bp, Artificial
  Synthetic probe AG9393_28_29
tgctttgttttaattaaacagtcggattcccctggtccgcaccagttcta

SEQ ID NO: 68 - DNA, 50 bp, Artificial
  Synthetic probe AG9394_28_30
agtcggctgctaggcgccggccgaggcgaggcgcgcgcggaaccgcggcc

SEQ ID NO: 69 - DNA, 49 bp, Artificial
  Synthetic probe AG9395_28_31
ccgggggcggacccggcggggggaccggcccgcggcccctccgccgcct

SEQ ID NO: 70 - DNA, 50 bp, Artificial
  Synthetic probe AG9396_28_32
gccgccgccgccgccgcgcgccgaggaggaggggggaacggggggcggac

SEQ ID NO: 71 - DNA, 48 bp, Artificial
  Synthetic probe AG9397_28_33
gggccggggggtagggcggggggacgaaccgccccgccccgccgcccg

SEQ ID NO: 72 - DNA, 50 bp, Artificial
  Synthetic probe AG9398_28_34
ccgaccgccgccgcccgaccgctcccgcccccagcggacgcgcgcgcgac

SEQ ID NO: 73 - DNA, 50 bp, Artificial
  Synthetic probe AG9399_28_35
cgagacgtggggtgggggtggggggcgcgccgcgccgccgccgggctccc

SEQ ID NO: 74 - DNA, 50 bp, Artificial
  Synthetic probe AG9400_28_36
cgggggcggccgcgacgcccgccgcagctggggcgatccacgggaagggc

SEQ ID NO: 75 - DNA, 50 bp, Artificial
  Synthetic probe AG9401_28_37
ccggctcgcgtccagagtccgcgccgccgccggccccccgggtccccggg

SEQ ID NO: 76 - DNA, 50 bp, Artificial
  Synthetic probe AG9402_28_38
gcccccctcgcggggacctgcccccgccggccgccccggcggccgccgcg

SEQ ID NO: 77 - DNA, 50 bp, Artificial
  Synthetic probe AG9403_28_39
cggcccctgccgccccgacccttctccccccgccgcgcccccacgcggcg

SEQ ID NO: 78 - DNA, 50 bp, Artificial
  Synthetic probe AG9404_28_40
ctcccccggggaggggggaggacggggagcgggggagagagagagagaga

SEQ ID NO: 79 - DNA, 50 bp, Artificial
  Synthetic probe AG9405_28_41
gggcgcggggtggggagggagcgagcggcgcgcgcgggtggggcggggga

SEQ ID NO: 80 - DNA, 49 bp, Artificial
  Synthetic probe AG9406_28_42
gggccgcgaggggggtgccccgggcgtgggggggcgcgcgcctcgtcca

SEQ ID NO: 81 - DNA, 50 bp, Artificial
  Synthetic probe AG9407_28_43
gccgcggcgcgcgcccagccccgcttcgcgccccagcccgaccgacccag

SEQ ID NO: 82 - DNA, 50 bp, Artificial
  Synthetic probe AG9408_28_44
cccttagagccaatccttatcccgaagttacggatccggcttgccgactt

SEQ ID NO: 83 - DNA, 50 bp, Artificial
  Synthetic probe AG9409_28_45
cccttacctacattgttccaacatgccagaggctgttcaccttggagacc

SEQ ID NO: 84 - DNA, 50 bp, Artificial
  Synthetic probe AG9410_28_46
tgctgcggatatgggtacggcccggcgcgagatttacaccctctcccccg

SEQ ID NO: 85 - DNA, 50 bp, Artificial
  Synthetic probe AG9411_28_47
gattttcaagggccagcgagagctcaccggacgccgccggaaccgcgacg

SEQ ID NO: 86 - DNA, 50 bp, Artificial
  Synthetic probe AG9412_28_48
ctttccaaggcacgggcccctctctcggggcgaacccattccagggcgcc

SEQ ID NO: 87 - DNA, 50 bp, Artificial
  Synthetic probe AG9413_28_49
ctgcccttcacaaagaaaagagaactctccccggggctcccgccggcttc

SEQ ID NO: 88 - DNA, 50 bp, Artificial
  Synthetic probe AG9414_28_50
tccgggatcggtcgcgttaccgcactggacgcctcgcggcgcccatctcc

SEQ ID NO: 89 - DNA, 50 bp, Artificial
  Synthetic probe AG9415_28_51
gccactccggattcggggatctgaacccgactccctttcgatcggccgag

SEQ ID NO: 90 - DNA, 50 bp, Artificial
  Synthetic probe AG9416_28_52
ggcaacggaggccatcgcccgtcccttcggaacggcgctcgcccatctct

SEQ ID NO: 91 - DNA, 50 bp, Artificial
  Synthetic probe AG9417_28_53
caggaccgactgacccatgttcaactgctgttcacatggaacccttctcc

SEQ ID NO: 92 - DNA, 50 bp, Artificial
  Synthetic probe AG9418_28_54
acttcggccttcaaagttctcgtttgaatatttgctactaccaccaagat

SEQ ID NO: 93 - DNA, 50 bp, Artificial
  Synthetic probe AG9419_28_55
ctgcacctgcggcggctccacccgggcccgcgccctaggcttcaaggctc

SEQ ID NO: 94 - DNA, 50 bp, Artificial
  Synthetic probe AG9420_28_56
accgcagcggccctcctactcgtcgcggcgtagcgtccgcggggctccgg

SEQ ID NO: 95 - DNA, 45 bp, Artificial
  Synthetic probe AG9421_28_57
gggcggggagcggggcgtgggcgggaggaggggaggaggcgtggg

SEQ ID NO: 96 - DNA, 50 bp, Artificial
  Synthetic probe AG9422_28_58
gggcgggggaaggaccccacacccccgccgccgccgccgccgccgccctc

SEQ ID NO: 97 - DNA, 50 bp, Artificial
  Synthetic probe AG9423_28_59
cgacgcacaccacacgcgcgcgcgcgcgcgccgcccccgccgctcccgtc

SEQ ID NO: 98 - DNA, 50 bp, Artificial
  Synthetic probe AG9424_28_60
cactctcgactgccggcgacggccgggtatgggcccgacgctccagcgcc

SEQ ID NO: 99 - DNA, 50 bp, Artificial
  Synthetic probe AG9425_28_61
atccattttcagggctagttgattcggcaggtgagttgttacacactcct

SEQ ID NO: 100 - DNA, 50 bp, Artificial
  Synthetic probe AG9426_28_62
tagcggattccgacttccatggccaccgtcctgctgtctatatcaaccaa

SEQ ID NO: 101 - DNA, 50 bp, Artificial
  Synthetic probe AG9427_28_63
caccttttctggggtctgatgagcgtcggcatcgggcgccttaacccggc

SEQ ID NO: 102 - DNA, 50 bp, Artificial
  Synthetic probe AG9428_28_64
gttcggttcatcccgcagcgccagttctgcttaccaaaagtggcccacta

SEQ ID NO: 103 - DNA, 50 bp, Artificial
  Synthetic probe AG9429_28_65
ggcactcgcattccacgcccggctccacgccagcgagccgggcttcttac

SEQ ID NO: 104 - DNA, 50 bp, Artificial
  Synthetic probe AG9430_28_66
ccatttaaagtttgagaataggttgagatcgtttcggccccaagacctct

SEQ ID NO: 105 - DNA, 50 bp, Artificial
  Synthetic probe AG9431_28_67
aatcattcgctttaccggataaaactgcgtggcgggggtgcgtcgggtct

SEQ ID NO: 106 - DNA, 50 bp, Artificial
  Synthetic probe AG9432_28_68
gcgagagcgccagctatcctgagggaaacttcggagggaaccagctacta

SEQ ID NO: 107 - DNA, 50 bp, Artificial
  Synthetic probe AG9433_28_69
gatggttcgattagtctttcgcccctatacccaggtcggacgaccgattt

SEQ ID NO: 108 - DNA, 50 bp, Artificial
  Synthetic probe AG9434_28_70
gcacgtcaggaccgctacggacctccaccagagtttcctctggcttcgcc

SEQ ID NO: 109 - DNA, 50 bp, Artificial
  Synthetic probe AG9435_28_71
ctgcccaggcatagttcaccatctttcgggtcctaacacgtgcgctcgtg

SEQ ID NO: 110 - DNA, 50 bp, Artificial
  Synthetic probe AG9436_28_72
ctccacctccccggcgcggcgggcgagacgggccggtggtgcgccctcgg

SEQ ID NO: 111 - DNA, 50 bp, Artificial
  Synthetic probe AG9437_28_73
cggactggagaggcctcgggatcccacctcggccggcgagcgcgccggcc

SEQ ID NO: 112 - DNA, 50 bp, Artificial
  Synthetic probe AG9438_28_74
ttcaccttcattgcgccacggcggctttcgtgcgagcccccgactcgcgc

SEQ ID NO: 113 - DNA, 50 bp, Artificial
  Synthetic probe AG9439_28_75
acgtgttagactccttggtccgtgtttcaagacgggtcgggtgggtagcc

SEQ ID NO: 114 - DNA, 49 bp, Artificial
  Synthetic probe AG9440_28_76
gacgtcgccgccgaccccgtgcgctcgctccgccgtccccctcttcggg

SEQ ID NO: 115 - DNA, 50 bp, Artificial
  Synthetic probe AG9441_28_77
gacgcgcgcgtggccccgagagaacctcccccgggcccgacggcgcgacc

SEQ ID NO: 116 - DNA, 50 bp, Artificial
  Synthetic probe AG9442_28_78
cgcccggggcgcactggggacagtccgccccgccccccgacccgcgcgcg

SEQ ID NO: 117 - DNA, 50 bp, Artificial
  Synthetic probe AG9443_28_79
gcaccccccccgtcgccggggcgggggcgcggggaggaggggtgggagag

SEQ ID NO: 118 - DNA, 50 bp, Artificial
  Synthetic probe AG9444_28_80
cggtcgcgccgtgggaggggtggcccggcccccccacgaggagacgccgg

SEQ ID NO: 119 - DNA, 50 bp, Artificial
  Synthetic probe AG9445_28_81
cgcgcccccgcgggggagacccccctcgcgggggattccccgcgggggtg

SEQ ID NO: 120 - DNA, 50 bp, Artificial
  Synthetic probe AG9446_28_82
ggcgccgggaggggggagagcgcggcgacgggtctcgctccctcggcccc

SEQ ID NO: 121 - DNA, 49 bp, Artificial
  Synthetic probe AG9447_28_83
gggattcggcgagtgctgctgccgggggggctgtaacactcgggggggt

SEQ ID NO: 122 - DNA, 50 bp, Artificial
  Synthetic probe AG9448_28_84
ttcggtcccgccgcccccgccgccgccgccaccgccgccgccgccgccgc

SEQ ID NO: 123 - DNA, 50 bp, Artificial
  Synthetic probe AG9449_28_85
cccgacccgcgcgccctcccgagggaggacgcggggccggggggcggaga

SEQ ID NO: 124 - DNA, 50 bp, Artificial
  Synthetic probe AG9450_28_86
cgggggaggaggaggacggacggacggacggggccccccgagccaccttc

SEQ ID NO: 125 - DNA, 50 bp, Artificial
  Synthetic probe AG9451_28_87
cccgccgggccttcccagccgtcccggagccggtcgcggcgcaccgccgc

SEQ ID NO: 126 - DNA, 50 bp, Artificial
  Synthetic probe AG9452_28_88
ggtggaaatgcgcccggcggcggccggtcgccggtcgggggacggtcccc

SEQ ID NO: 127 - DNA, 50 bp, Artificial
  Synthetic probe AG9453_28_89
cgccgaccccacccccggccccgcccgcccacccccgcacccgccggagc

SEQ ID NO: 128 - DNA, 50 bp, Artificial
  Synthetic probe AG9454_28_90
ccgccccctccggggaggaggaggaggggcggcgggggaagggagggcgg

SEQ ID NO: 129 - DNA, 50 bp, Artificial
  Synthetic probe AG9455_28_91
gtggaggggtcgggaggaacggggggcgggaaagatccgccgggccgccg

SEQ ID NO: 130 - DNA, 50 bp, Artificial
  Synthetic probe AG9456_28_92
acacggccggacccgccgccgggttgaatcctccgggcggactgcgcgga

SEQ ID NO: 131 - DNA, 50 bp, Artificial
  Synthetic probe AG9457_28_93
ccccacccgtttacctcttaacggtttcacgccctcttgaactctctctt

SEQ ID NO: 132 - DNA, 50 bp, Artificial
  Synthetic probe AG9458_28_94
caaagttcttttcaactttcccttacggtacttgttgactatcggtctcg

SEQ ID NO: 133 - DNA, 50 bp, Artificial
  Synthetic probe AG9459_28_95
tgccggtatttagccttagatggagtttaccacccgctttgggctgcatt

SEQ ID NO: 134 - DNA, 50 bp, Artificial
  Synthetic probe AG9460_28_96
cccaagcaacccgactccgggaagacccgggcgcgcgccggccgctaccg

SEQ ID NO: 135 - DNA, 50 bp, Artificial
  Synthetic probe AG9461_28_97
gcctcacaccgtccacgggctgggcctcgatcagaaggacttgggccccc

SEQ ID NO: 136 - DNA, 50 bp, Artificial
  Synthetic probe AG9462_28_98
cacgagcggcgccggggagcgggtcttccgtacgccacatgtcccgcgcc

SEQ ID NO: 137 - DNA, 50 bp, Artificial
  Synthetic probe AG9463_28_99
ccgcggggcggggattcggcgctgggctcttccctgttcactcgccgtta

SEQ ID NO: 138 - DNA, 50 bp, Artificial
  Synthetic probe AG9464_28_100
ctgagggaatcctggttagtttcttttcctccgctgactaatatgcttaa

SEQ ID NO: 139 - DNA, 50 bp, Artificial
  Synthetic probe AG9465_28_101
gactaatatgcttaaattcagcgggtcgccacgtctgatctgaggtcgcg

SEQ ID NO: 140 - DNA, 50 bp, Artificial
  Synthetic probe AG9466_5.8_1
aagcgacgctcagacaggcgtagccccgggaggaacccggggccgcaagt

SEQ ID NO: 141 - DNA, 50 bp, Artificial
  Synthetic probe AG9467_5.8_2
gcgttcgaagtgtcgatgatcaatgtgtcctgcaattcacattaattctc

SEQ ID NO: 142 - DNA, 50 bp, Artificial
  Synthetic probe AG9468_5.8_3
gcagctagctgcgttcttcatcgacgcacgagccgagtgatccaccgcta

SEQ ID NO: 143 - DNA, 50 bp, Artificial
  Synthetic probe AG9469_16_1
aaaccctgttcttgggtgggtgtgggtataatactaagttgagatgatat

SEQ ID NO: 144 - DNA, 50 bp, Artificial
  Synthetic probe AG9470_16_2
catttacgggggaaggcgctttgtgaagtaggccttatttctcttgtcct

SEQ ID NO: 145 - DNA, 50 bp, Artificial
  Synthetic probe AG9471_16_3
  misc_feature (23)..(23): n is a, c, g, or t
ttcgtacagggaggaatttgaangtagatagaaaccgacctggattactc

SEQ ID NO: 146 - DNA, 50 bp, Artificial
  Synthetic probe AG9472_16_4
cggtctgaactcagatcacgtaggactttaatcgttgaacaaacgaacct

SEQ ID NO: 147 - DNA, 50 bp, Artificial
  Synthetic probe AG9473_16_5
ttaatagcggctgcaccatcgggatgtcctgatccaacatcgaggtcgta

SEQ ID NO: 148 - DNA, 50 bp, Artificial
  Synthetic probe AG9474_16_6
aaccctattgttgatatggactctagaataggattgcgctgttatcccta

SEQ ID NO: 149 - DNA, 50 bp, Artificial
  Synthetic probe AG9475_16_7
gggtaacttgttccgttggtcaagttattggatcaattgagtatagtagt

SEQ ID NO: 150 - DNA, 50 bp, Artificial
  Synthetic probe AG9476_16_8
tcgctttgactggtgaagtcttagcatgtactgctcggaggttgggttct

SEQ ID NO: 151 - DNA, 50 bp, Artificial
  Synthetic probe AG9477_16_9
gctccgaggtcgccccaaccgaaatttttaatgcaggtttggtagtttag

SEQ ID NO: 152 - DNA, 50 bp, Artificial
  Synthetic probe AG9478_16_10
gacctgtgggtttgttaggtactgtttgcattaataaattaaagctccat

SEQ ID NO: 153 - DNA, 50 bp, Artificial
  Synthetic probe AG9479_16_11
agggtcttctcgtcttgctgtgttatgcccgcctcttcacgggcaggtca

SEQ ID NO: 154 - DNA, 50 bp, Artificial
  Synthetic probe AG9480_16_12
atttcactggttaaaagtaagagacagctgaaccctcgtggagccattca

SEQ ID NO: 155 - DNA, 50 bp, Artificial
  Synthetic probe AG9481_16_13
tacaggtccctatttaaggaacaagtgattatgctacctttgcacggtta

SEQ ID NO: 156 - DNA, 50 bp, Artificial
  Synthetic probe AG9482_16_14
gggtaccgcggccgttaaacatgtgtcactgggcaggcggtgcctctaat

SEQ ID NO: 157 - DNA, 50 bp, Artificial
  Synthetic probe AG9483_16_15
actggtgatgctagaggtgatgtttttggtaaacaggcggggtaagattt

SEQ ID NO: 158 - DNA, 50 bp, Artificial
  Synthetic probe AG9484_16_16
gccgagttccttttactttttttaacctttccttatgagcatgcctgtgt

SEQ ID NO: 159 - DNA, 50 bp, Artificial
  Synthetic probe AG9485_16_17
tgggttgacagtgagggtaataatgacttgttggttgattgtagatattg

SEQ ID NO: 160 - DNA, 50 bp, Artificial
  Synthetic probe AG9486_16_18
ggctgttaattgtcagttcagtgttttaatctgacgcaggcttatgcgga

SEQ ID NO: 161 - DNA, 50 bp, Artificial
  Synthetic probe AG9487_16_19
ggagaatgttttcatgttacttatactaacattagttcttctatagggtg

SEQ ID NO: 162 - DNA, 50 bp, Artificial
  Synthetic probe AG9488_16_20
atagattggtccaattgggtgtgaggagttcagttatatgtttgggattt

SEQ ID NO: 163 - DNA, 50 bp, Artificial
  Synthetic probe AG9489_16_21
tttaggtagtgggtgttgagcttgaacgctttcttaattggtggctgctt

SEQ ID NO: 164 - DNA, 50 bp, Artificial
  Synthetic probe AG9490_16_22
ttaggcctactatgggtgttaaattttttactctctctacaaggtttttt

SEQ ID NO: 165 - DNA, 50 bp, Artificial
  Synthetic probe AG9491_16_23
cctagtgtccaaagagctgttcctctttggactaacagttaaatttacaa

SEQ ID NO: 166 - DNA, 49 bp, Artificial
  Synthetic probe AG9492_16_24
gggatttagagggttctgtgggcaaatttaaagttgaactaagattcta

SEQ ID NO: 167 - DNA, 50 bp, Artificial
  Synthetic probe AG9493_16_25
tcttggacaaccagctatcaccaggctcggtaggtttgtcgcctctacct

SEQ ID NO: 168 - DNA, 50 bp, Artificial
  Synthetic probe AG9494_16_26
ataaatcttcccactattttgctacatagacgggtgtgctcttttagctg

SEQ ID NO: 169 - DNA, 50 bp, Artificial
  Synthetic probe AG9495_16_27
ttcttaggtagctcgtctggtttcgggggtcttagctttggctctccttg

SEQ ID NO: 170 - DNA, 50 bp, Artificial
  Synthetic probe AG9496_16_28
caaagttatttctagttaattcattatgcagaaggtataggggttagtcc

SEQ ID NO: 171 - DNA, 50 bp, Artificial
  Synthetic probe AG9497_16_29
ttgctatattatgcttggttataatttttcatctttcccttgcggtacta

SEQ ID NO: 172 - DNA, 50 bp, Artificial
  Synthetic probe AG9498_16_30
tatctattgcgccaggtttcaatttctatcgcctatactttatttgggta

SEQ ID NO: 173 - DNA, 50 bp, Artificial
  Synthetic probe AG9499_16_31
aatggtttggctaaggttgtctggtagtaaggtggagtgggtttggggct

SEQ ID NO: 174 - DNA, 50 bp, Artificial
  Synthetic probe AG9500_12_1
gttcgtccaagtgcactttccagtacacttaccatgttacgacttgtctc

SEQ ID NO: 175 - DNA, 50 bp, Artificial
  Synthetic probe AG9501_12_2
ctctatataaatgcgtaggggttttagttaaatgtcctttgaagtatact

SEQ ID NO: 176 - DNA, 50 bp, Artificial
  Synthetic probe AG9502_12_3
tgaggagggtgacgggcggtgtgtacgcgcttcagggccctgttcaacta

SEQ ID NO: 177 - DNA, 50 bp, Artificial
  Synthetic probe AG9503_12_4
agcactctactcttagtttactgctaaatccaccttcgacccttaagttt

SEQ ID NO: 178 - DNA, 50 bp, Artificial
  Synthetic probe AG9504_12_5
cataagggctatcgtagttttctggggtagaaaatgtagcccatttcttg

SEQ ID NO: 179 - DNA, 50 bp, Artificial
  Synthetic probe AG9505_12_6
ccacctcatgggctacaccttgacctaacgtctttacgtgggtacttgcg

SEQ ID NO: 180 - DNA, 50 bp, Artificial
  Synthetic probe AG9506_12_7
cttactttgtagccttcatcagggtttgctgaagatggcggtatataggc

SEQ ID NO: 181 - DNA, 50 bp, Artificial
  Synthetic probe AG9507_12_8
tgagcaagaggtggtgaggttgatcggggtttatcgattacagaacaggc

SEQ ID NO: 182 - DNA, 50 bp, Artificial
  Synthetic probe AG9508_12_9
tcctctagagggatatgaagcaccgccaggtcctttgagttttaagctgt

SEQ ID NO: 183 - DNA, 50 bp, Artificial
  Synthetic probe AG9509_12_10
ggctcgtagtgttctggcgagcagttttgttgatttaactgttgaggttt

SEQ ID NO: 184 - DNA, 50 bp, Artificial
  Synthetic probe AG9510_12_11
agggctaagcatagtggggtatctaatcccagtttgggtcttagctattg

SEQ ID NO: 185 - DNA, 50 bp, Artificial
  Synthetic probe AG9511_12_12
tgtgttcagatatgttaaagccactttcgtagtctattttgtgtcaactg

SEQ ID NO: 186 - DNA, 50 bp, Artificial
  Synthetic probe AG9512_12_13
gagttttttacaactcaggtgagttttagctttattggggagggggtgat

SEQ ID NO: 187 - DNA, 50 bp, Artificial
  Synthetic probe AG9513_12_14
ctaaaacactctttacgccggcttctattgacttgggttaatcgtgtgac

SEQ ID NO: 188 - DNA, 50 bp, Artificial
  Synthetic probe AG9514_12_15
cgcggtggctggcacgaaattgaccaaccctggggttagtatagcttagt

SEQ ID NO: 189 - DNA, 48 bp, Artificial
  Synthetic probe AG9515_12_16
taaactttcgtttattgctaaaggttaatcactgctgtttcccgtggg

SEQ ID NO: 190 - DNA, 50 bp, Artificial
  Synthetic probe AG9516_12_17
tgtggctaggctaagcgttttgagctgcattgctgcgtgcttgatgcttg

SEQ ID NO: 191 - DNA, 50 bp, Artificial
  Synthetic probe AG9517_12_18
ttccttttgatcgtggtgatttagagggtgaactcactggaacggggatg

SEQ ID NO: 192 - DNA, 50 bp, Artificial
  Synthetic probe AG9518_12_19
cttgcatgtgtaatcttactaagagctaatagaaaggctaggaccaaacc

SEQ ID NO: 193 - DNA, 50 bp, Artificial
  Synthetic probe AG9519_5_1
aaagcctacagcacccggtattcccaggcggtctcccatccaagtactaa

SEQ ID NO: 194 - DNA, 50 bp, Artificial
  Synthetic probe AG9520_5_2
ccaggcccgaccctgcttagcttccgagatcagacgagatcgggcgcgtt

SEQ ID NO: 195 - DNA, 50 bp, Artificial
  Synthetic probe AG9521_5_3
ttccgagatcagacgagatcgggcgcgttcagggtggtatggccgtagac